European Patent Application EP 4 431 102 A1, published September 18, 2024. Title: Compositions for removing senescent cells and uses thereof. Applicant: Lifeceutix Co., Ltd. The sequence listing filed with the application follows.

SEQUENCE LISTING (40 sequences)

SEQ ID NO: 1 - DNA, 20 bp, synthetic construct
  source 1..20: mol_type = other DNA
ggaagggctcatgaccacag

SEQ ID NO: 2 - DNA, 21 bp, synthetic construct
  source 1..21: mol_type = other DNA
acagtcttctgggtggcagtg

SEQ ID NO: 3 - DNA, 20 bp, synthetic construct
  source 1..20: mol_type = other DNA
tgagctttggttctgccatt

SEQ ID NO: 4 - DNA, 21 bp, synthetic construct
  source 1..21: mol_type = other DNA
agctgtcgacttcatgacaag

SEQ ID NO: 5 - DNA, 24 bp, synthetic construct
  source 1..24: mol_type = other DNA
gagactaaggcagaagatgtagag

SEQ ID NO: 6 - DNA, 19 bp, synthetic construct
  source 1..19: mol_type = other DNA
gcagaccagcatgacagat

SEQ ID NO: 7 - DNA, 21 bp, synthetic construct
  source 1..21: mol_type = other DNA
gtgaagaagaggacagcactg

SEQ ID NO: 8 - DNA, 18 bp, synthetic construct
  source 1..18: mol_type = other DNA
cccattcccaccatcacc

SEQ ID NO: 9 - DNA, 23 bp, synthetic construct
  source 1..23: mol_type = other DNA
aagggacacagaggtttcagtgg

SEQ ID NO: 10 - DNA, 24 bp, synthetic construct
  source 1..24: mol_type = other DNA
cagcaccagtagcaccatcatttc

SEQ ID NO: 11 - DNA, 24 bp, synthetic construct
  source 1..24: mol_type = other DNA
cttgcagtaaccttatgcctagca

SEQ ID NO: 12 - DNA, 25 bp, synthetic construct
  source 1..25: mol_type = other DNA
cccatctaacctctctacccagtct

SEQ ID NO: 13 - DNA, 20 bp, synthetic construct
  source 1..20: mol_type = other DNA
tgtcagtcaaagcaagcccg

SEQ ID NO: 14 - DNA, 24 bp, synthetic construct
  source 1..24: mol_type = other DNA
ttaggacgctcataagtgtcaccc

SEQ ID NO: 15 - DNA, 25 bp, synthetic construct
  source 1..25: mol_type = other DNA
catccgtaaagacctctatgccaac

SEQ ID NO: 16 - DNA, 19 bp, synthetic construct
  source 1..19: mol_type = other DNA
atggagccaccgatccaca

SEQ ID NO: 17 - DNA, 21 bp, synthetic construct
  source 1..21: mol_type = other DNA
gcagatccacagcgatatcca

SEQ ID NO: 18 - DNA, 20 bp, synthetic construct
  source 1..20: mol_type = other DNA
aacaggtcggacatcaccag

SEQ ID NO: 19 - DNA, 21 bp, synthetic construct
  source 1..21: mol_type = other DNA
tccataacccatgatctggaa

SEQ ID NO: 20 - DNA, 21 bp, synthetic construct
  source 1..21: mol_type = other DNA
ttggttgagggaatcattcat

SEQ ID NO: 21 - DNA, 19 bp, synthetic construct
  source 1..19: mol_type = other DNA
gtatgggctggactgtttc

SEQ ID NO: 22 - DNA, 18 bp, synthetic construct
  source 1..18: mol_type = other DNA
gctgtctgctcattcacg

SEQ ID NO: 23 - DNA, 21 bp, synthetic construct
  source 1..21: mol_type = other DNA
accgaagtcatagccacactc

SEQ ID NO: 24 - DNA, 20 bp, synthetic construct
  source 1..20: mol_type = other DNA
ctccgttacttggggacacc

SEQ ID NO: 25 - DNA, 18 bp, synthetic construct
  source 1..18: mol_type = other DNA
gctgccgtcattttctgc

SEQ ID NO: 26 - DNA, 18 bp, synthetic construct
  source 1..18: mol_type = other DNA
tctcactggcccgtcatc

SEQ ID NO: 27 - DNA, 23 bp, synthetic construct
  source 1..23: mol_type = other DNA
gttggagaacatggagactttgt

SEQ ID NO: 28 - DNA, 21 bp, synthetic construct
  source 1..21: mol_type = other DNA
caagttcatgagcagcaacca

SEQ ID NO: 29 - DNA, 22 bp, synthetic construct
  source 1..22: mol_type = other DNA
tgcactctgctgaaaggagtct

SEQ ID NO: 30 - DNA, 24 bp, synthetic construct
  source 1..24: mol_type = other DNA
gtcattggaattctgtcctttcca

SEQ ID NO: 31 - DNA, 22 bp, synthetic construct
  source 1..22: mol_type = other DNA
aaggggataacagccactacaa

SEQ ID NO: 32 - DNA, 25 bp, synthetic construct
  source 1..25: mol_type = other DNA
accaacataaaaattaagccaaatg

SEQ ID NO: 33 - DNA, 21 bp, synthetic construct
  source 1..21: mol_type = other DNA
gcatctgccctaaggtcttca

SEQ ID NO: 34 - DNA, 23 bp, synthetic construct
  source 1..23: mol_type = other DNA
gtggaaaaggtagtggatgcatt

SEQ ID NO: 35 - DNA, 21 bp, synthetic construct
  source 1..21: mol_type = other DNA
cagtcgattcacctacagcac

SEQ ID NO: 36 - DNA, 17 bp, synthetic construct
  source 1..17: mol_type = other DNA
tggagggagtttacacg

SEQ ID NO: 37 - DNA, 20 bp, synthetic construct
  source 1..20: mol_type = other DNA
aagggccattttgcttttct

SEQ ID NO: 38 - DNA, 20 bp, synthetic construct
  source 1..20: mol_type = other DNA
aactcacagcaaccctccaa

SEQ ID NO: 39 - DNA, 19 bp, synthetic construct
  source 1..19: mol_type = other DNA
tgccagagccaacgtcaag

SEQ ID NO: 40 - DNA, 20 bp, synthetic construct
  source 1..20: mol_type = other DNA
cagccgggctacaatctgaa